European Patent Application EP 4 389 913 A1, published June 26, 2024. Title: A PCR-ELISA analogous antibody-free method for detecting a target nucleic acid in a sample. Applicant: Universität Heidelberg. The sequence listing filed with the application follows.

SEQUENCE LISTING (30 sequences)

SEQ ID NO: 1 - protein, 212 aa, Carica papaya
  source 1..212: note = PAPA1_CARPA
IPEYVDWRQKGAVTPVKNQGSCGSCWAFSAVVTIEGIIKIRTGNLNEYSEQELLDCDRRSYGCNGGYPWSALQLVAQYGIHYRNTYPYEGVQRYCRSREKGPYAAKTDGVRQVQPYNEGALLYSIANQPVSVVLEAAGKDFQLYRGGIFVGPCGNKVDHAVAAVGYGPNYILIKNSWGTGWGENGYIRIKRGTGNSYGVCGLYTSSFYPVKN

SEQ ID NO: 2 - protein, 345 aa, Carica papaya
  source 1..345: note = papain precursor protein contains 345 amino acid residues
MAMIPSISKLLFVAICLFVYMGLSFGDFSIVGYSQNDLTSTERLIQLFESWMLKHNKIYKNIDEKIYRFEIFKDNLKYIDETNKKNNSYWLGLNVFADMSNDEFKEKYTGSIAGNYTTTELSYEEVLNDGDVNIPEYVDWRQKGAVTPVKNQGSCGSCWAFSAVVTIEGIIKIRTGNLNEYSEQELLDCDRRSYGCNGGYPWSALQLVAQYGIHYRNTYPYEGVQRYCRSREKGPYAAKTDGVRQVQPYNEGALLYSIANQPVSVVLEAAGKDFQLYRGGIFVGPCGNKVDHAVAAVGYGPNYILIKNSWGTGWGENGYIRIKRGTGNSYGVCGLYTSSFYPVKN

SEQ ID NO: 3 - protein, 19 aa, Carica papaya
  source 1..19: note = signal sequence of papain
MAMIPSISKLLFVAICLFV

SEQ ID NO: 4 - protein, 133 aa, Carica papaya
  source 1..133: note = propeptide of papain
YMGLSFGDFSIVGYSQNDLTSTERLIQLFESWMLKHNKIYKNIDEKIYRFEIFKDNLKYIDETNKKNNSYWLGLNVFADMSNDEFKEKYTGSIAGNYTTTELSYEEVLNDGDVNIPEYVDWRQKGAVTPVKNQ

SEQ ID NO: 5 - protein, 4 aa, synthetic construct
  source 1..4: note = peptide of the invention
CCRG

SEQ ID NO: 6 - protein, 4 aa, synthetic construct
  source 1..4: note = peptide of the invention
CEWG

SEQ ID NO: 7 - protein, 5 aa, synthetic construct
  source 1..5: note = peptide of the invention
CGGGG

SEQ ID NO: 8 - protein, 4 aa, synthetic construct
  source 1..4: note = peptide of the invention
CKSG

SEQ ID NO: 9 - protein, 4 aa, synthetic construct
  source 1..4: note = peptide of the invention
CLCG

SEQ ID NO: 10 - protein, 5 aa, synthetic construct
  source 1..5: note = peptide of the invention
CLRCG

SEQ ID NO: 11 - protein, 4 aa, synthetic construct
  source 1..4: note = peptide of the invention
CLRG

SEQ ID NO: 12 - protein, 4 aa, synthetic construct
  source 1..4: note = peptide of the invention
CSGG

SEQ ID NO: 13 - protein, 4 aa, synthetic construct
  source 1..4: note = peptide of the invention
CVQG

SEQ ID NO: 14 - protein, 4 aa, synthetic construct
  source 1..4: note = peptide of the invention
CWRG

SEQ ID NO: 15 - protein, 6 aa, synthetic construct
  source 1..6: note = peptide of the invention
EGCGRG

SEQ ID NO: 16 - protein, 4 aa, synthetic construct
  source 1..4: note = peptide of the invention
FCLR

SEQ ID NO: 17 - protein, 6 aa, synthetic construct
  source 1..6: note = peptide of the invention
FVCEKG

SEQ ID NO: 18 - protein, 6 aa, synthetic construct
  source 1..6: note = peptide of the invention
GGCGGG

SEQ ID NO: 19 - protein, 6 aa, synthetic construct
  source 1..6: note = peptide of the invention
GKCLRG

SEQ ID NO: 20 - protein, 6 aa, synthetic construct
  source 1..6: note = peptide of the invention
GLCLRG

SEQ ID NO: 21 - protein, 6 aa, synthetic construct
  source 1..6: note = peptide of the invention
SECLRG

SEQ ID NO: 22 - protein, 4 aa, synthetic construct
  source 1..4: note = peptide of the invention
VCLR

SEQ ID NO: 23 - protein, 4 aa, synthetic construct
  source 1..4: note = peptide of the invention
YCLR

SEQ ID NO: 24 - protein, 6 aa, synthetic construct
  source 1..6: note = peptide of the invention
YWCLVG

SEQ ID NO: 25 - DNA, 968 bp, synthetic construct
  source 1..968: mol_type = other DNA; note = SARS-CoV-2-S-RBD-sfGFP plasmid
cagagctctctggctaactagagaacccactgcttactggcttatcgaaattaatacgactcactatagggagacccaagctggctagcgccaccatgaagaccatcatcgccctgagctacatcttctgcctggtgttcgccactaatctttgtccgttcggtgaggtttttaacgcgacaaggttcgctagtgtatatgcttggaaccgaaagagaatctccaattgcgtagctgattactccgttctctataacagtgcgtccttttcaacctttaagtgttacggcgtttctccaacgaagctgaatgatctctgttttacgaacgtgtatgctgactctttcgttatacggggggacgaagtgagacagatagcaccaggtcagactgggaagatagcggattacaactataagttgcccgatgattttacggggtgcgtaatcgcatggaactcaaacaacctcgactccaaagtaggtggtaattataattacttgtatcgcctgtttcgaaagagcaatttgaagccttttgagcgggatatttcaaccgaaatttaccaagcaggcagtacgccatgtaacggagtagagggatttaattgctactttcctcttcaatcttatggctttcaaccaacaaacggagtggggtatcaaccttatagagtggtagtattgtcctttgagctcctccacgccccggctacagtttgtgggcccaaaaagggatccggtgggtccggtagtggtggttccaaaggagaagaacttttcactggagttgtcccaattcttgttgaattagatggtgatgttaatgggcacaaattttctgtccgtggagagggtgaaggtgatgctacaaacggaaaactcacccttaaatttatttgcactactggaaaactacctgttccatggccaacacttgtcactactctgacctatggtgttcaatgc

SEQ ID NO: 26 - DNA, 713 bp, synthetic construct
  source 1..713: mol_type = other DNA; note = T7-Spike full DNA
taatacgactcactatagggagacccaagctggctagcgccaccatgaagaccatcatcgccctgagctacatcttctgcctggtgttcgccactaatctttgtccgttcggtgaggtttttaacgcgacaaggttcgctagtgtatatgcttggaaccgaaagagaatctccaattgcgtagctgattactccgttctctataacagtgcgtccttttcaacctttaagtgttacggcgtttctccaacgaagctgaatgatctctgttttacgaacgtgtatgctgactctttcgttatacggggggacgaagtgagacagatagcaccaggtcagactgggaagatagcggattacaactataagttgcccgatgattttacggggtgcgtaatcgcatggaactcaaacaacctcgactccaaagtaggtggtaattataattacttgtatcgcctgtttcgaaagagcaatttgaagccttttgagcgggatatttcaaccgaaatttaccaagcaggcagtacgccatgtaacggagtagagggatttaattgctactttcctcttcaatcttatggctttcaaccaacaaacggagtggggtatcaaccttatagagtggtagtattgtcctttgagctcctccacgccccggctacagtttgtgggcccaaaaagggatccggtgggtccggtagtggtggttcc

SEQ ID NO: 27 - DNA, 669 bp, synthetic construct
  source 1..669: mol_type = other DNA; note = Spike full DNA
atgaagaccatcatcgccctgagctacatcttctgcctggtgttcgccactaatctttgtccgttcggtgaggtttttaacgcgacaaggttcgctagtgtatatgcttggaaccgaaagagaatctccaattgcgtagctgattactccgttctctataacagtgcgtccttttcaacctttaagtgttacggcgtttctccaacgaagctgaatgatctctgttttacgaacgtgtatgctgactctttcgttatacggggggacgaagtgagacagatagcaccaggtcagactgggaagatagcggattacaactataagttgcccgatgattttacggggtgcgtaatcgcatggaactcaaacaacctcgactccaaagtaggtggtaattataattacttgtatcgcctgtttcgaaagagcaatttgaagccttttgagcgggatatttcaaccgaaatttaccaagcaggcagtacgccatgtaacggagtagagggatttaattgctactttcctcttcaatcttatggctttcaaccaacaaacggagtggggtatcaaccttatagagtggtagtattgtcctttgagctcctccacgccccggctacagtttgtgggcccaaaaagggatccggtgggtccggtagtggtggttcc

SEQ ID NO: 28 - DNA, 20 bp, synthetic construct
  source 1..20: mol_type = other DNA; note = T7 forward
taatacgactcactataggg

SEQ ID NO: 29 - DNA, 17 bp, synthetic construct
  source 1..17: mol_type = other DNA; note = Spike forward
atgaagaccatcatcgc

SEQ ID NO: 30 - DNA, 15 bp, synthetic construct
  source 1..15: mol_type = other DNA; note = Spike reverse
ggaaccaccactacc